European Patent Application EP 4 261 232 A1, published October 18, 2023. Title: HUMAN PAPILLOMAVIRUS TYPE 18 CHIMERIC PROTEIN AND USE THEREOF. Applicant: Institute of Basic Medical Sciences Chinese Academy of Medical Sciences. The sequence listing filed with the application follows.

SEQUENCE LISTING (51 sequences)

SEQ ID NO: 1 - protein, 507 aa, HPV 18
MALWRPSDNTVYLPPPSVARVVNTDDYVTRTSIFYHAGSSRLLTVGNPYFRVPAGGGNKQDIPKVSAYQYRVFRVQLPDPNKFGLPDTSIYNPETQRLVWACAGVEIGRGQPLGVGLSGHPFYNKLDDTESSHAATSNVSEDVRDNVSVDYKQTQLCILGCAPAIGEHWAKGTACKSRPLSQGDCPPLELKNTVLEDGDMVDTGYGAMDFSTLQDTKCEVPLDICQSICKYPDYLQMSADPYGDSMFFCLRREQLFARHFWNRAGTMGDTVPQSLYIKGTGMRASPGSCVYSPSPSGSIVTSDSQLFNKPYWLHKAQGHNNGVCWHNQLFVTVVDTTRSTNLTICASTQSPVPGQYDATKFKQYSRHVEEYDLQFIFQLCTITLTADVMSYIHSMNSSILEDWNFGVPPPPTTSLVDTYRFVQSVAITCQKDAAPAENKDPYDKLKFWNVDLKEKFSLDLDQYPLGRKFLVQAGLRRKPTIGPRKRSAPSATTSSKPAKRVRVRARK

SEQ ID NO: 2 - protein, 464 aa, HPV 59
MVSHRAARRKRASATDLYKTCKQAGTCPSDVINKVEGTTLADKILQWTSLGIFLGGLGIGTGSGTGGRTGYIPLGGRTNTIVDVSPAKPPVVIEPVGPTDPSIVTLVEDSSVITSGAPAPTFTGTSGFEISTSSTTTPAVLDITPTSSVQISSSSFINPAFTDPSVIEVPQTGEISGNILISTPTSGAHGYEEIPMQTFATEGTGLEPISSTPNPTVRRVAGPRLYSRANQQVRVSDANFLTRPSTFVTYDNPAYDPIDTTLTFDPSSEVPDPDFMDIVRLHRPALTSRRSTVRFSRLGQRATMFTRSGKQIGARVHFYHDISPIPHAENIELQPLVSSQAATDDIYDIYADITDEAPTSTANTAFTIPKSSFQSLSLTRSASSTFSNVTVPLATAWDVPVNTGPDIVLPNTNIVGPTYSTTPFTTIQSINIEGTNYFLWPIYYFLPRKRKRVPYFFTDGSMAF

SEQ ID NO: 3 - protein, 21 aa, HPV 59
LYKTCKQAGTCPSDVINKVEG

SEQ ID NO: 4 - protein, 16 aa, HPV 59
LYKTCKQAGTCPSDVI

SEQ ID NO: 5 - protein, 20 aa, HPV 59
DLYKTCKQAGTCPSDVINKV

SEQ ID NO: 6 - protein, 22 aa, HPV 59
DLYKTCKQAGTCPSDVINKVEG

SEQ ID NO: 7 - protein, 523 aa, Artificial Sequence
  PEPTIDE (1)..(523): 18L1DE137-138/59dES
MALWRPSDNTVYLPPPSVARVVNTDDYVTRTSIFYHAGSSRLLTVGNPYFRVPAGGGNKQDIPKVSAYQYRVFRVQLPDPNKFGLPDTSIYNPETQRLVWACAGVEIGRGQPLGVGLSGHPFYNKLDDTESSHAATSLYKTCKQAGTCPSDVINVSEDVRDNVSVDYKQTQLCILGCAPAIGEHWAKGTACKSRPLSQGDCPPLELKNTVLEDGDMVDTGYGAMDFSTLQDTKCEVPLDICQSICKYPDYLQMSADPYGDSMFFCLRREQLFARHFWNRAGTMGDTVPQSLYIKGTGMRASPGSCVYSPSPSGSIVTSDSQLFNKPYWLHKAQGHNNGVCWHNQLFVTVVDTTRSTNLTICASTQSPVPGQYDATKFKQYSRHVEEYDLQFIFQLCTITLTADVMSYIHSMNSSILEDWNFGVPPPPTTSLVDTYRFVQSVAITCQKDAAPAENKDPYDKLKFWNVDLKEKFSLDLDQYPLGRKFLVQAGLRRKPTIGPRKRSAPSATTSSKPAKRVRVRARK

SEQ ID NO: 8 - protein, 491 aa, Artificial Sequence
  PEPTIDE (1)..(491): 18L1 delta CDE137-138/59dES
MALWRPSDNTVYLPPPSVARVVNTDDYVTRTSIFYHAGSSRLLTVGNPYFRVPAGGGNKQDIPKVSAYQYRVFRVQLPDPNKFGLPDTSIYNPETQRLVWACAGVEIGRGQPLGVGLSGHPFYNKLDDTESSHAATSLYKTCKQAGTCPSDVINVSEDVRDNVSVDYKQTQLCILGCAPAIGEHWAKGTACKSRPLSQGDCPPLELKNTVLEDGDMVDTGYGAMDFSTLQDTKCEVPLDICQSICKYPDYLQMSADPYGDSMFFCLRREQLFARHFWNRAGTMGDTVPQSLYIKGTGMRASPGSCVYSPSPSGSIVTSDSQLFNKPYWLHKAQGHNNGVCWHNQLFVTVVDTTRSTNLTICASTQSPVPGQYDATKFKQYSRHVEEYDLQFIFQLCTITLTADVMSYIHSMNSSILEDWNFGVPPPPTTSLVDTYRFVQSVAITCQKDAAPAENKDPYDKLKFWNVDLKEKFSLDLDQYPLGRKFLVQAGL

SEQ ID NO: 9 - protein, 527 aa, Artificial Sequence
  PEPTIDE (1)..(527): 18L1DE137-138/59dE
MALWRPSDNTVYLPPPSVARVVNTDDYVTRTSIFYHAGSSRLLTVGNPYFRVPAGGGNKQDIPKVSAYQYRVFRVQLPDPNKFGLPDTSIYNPETQRLVWACAGVEIGRGQPLGVGLSGHPFYNKLDDTESSHAATSDLYKTCKQAGTCPSDVINKVNVSEDVRDNVSVDYKQTQLCILGCAPAIGEHWAKGTACKSRPLSQGDCPPLELKNTVLEDGDMVDTGYGAMDFSTLQDTKCEVPLDICQSICKYPDYLQMSADPYGDSMFFCLRREQLFARHFWNRAGTMGDTVPQSLYIKGTGMRASPGSCVYSPSPSGSIVTSDSQLFNKPYWLHKAQGHNNGVCWHNQLFVTVVDTTRSTNLTICASTQSPVPGQYDATKFKQYSRHVEEYDLQFIFQLCTITLTADVMSYIHSMNSSILEDWNFGVPPPPTTSLVDTYRFVQSVAITCQKDAAPAENKDPYDKLKFWNVDLKEKFSLDLDQYPLGRKFLVQAGLRRKPTIGPRKRSAPSATTSSKPAKRVRVRARK

SEQ ID NO: 10 - protein, 495 aa, Artificial Sequence
  PEPTIDE (1)..(495): 18L1 delta CDE137-138/59dE
MALWRPSDNTVYLPPPSVARVVNTDDYVTRTSIFYHAGSSRLLTVGNPYFRVPAGGGNKQDIPKVSAYQYRVFRVQLPDPNKFGLPDTSIYNPETQRLVWACAGVEIGRGQPLGVGLSGHPFYNKLDDTESSHAATSDLYKTCKQAGTCPSDVINKVNVSEDVRDNVSVDYKQTQLCILGCAPAIGEHWAKGTACKSRPLSQGDCPPLELKNTVLEDGDMVDTGYGAMDFSTLQDTKCEVPLDICQSICKYPDYLQMSADPYGDSMFFCLRREQLFARHFWNRAGTMGDTVPQSLYIKGTGMRASPGSCVYSPSPSGSIVTSDSQLFNKPYWLHKAQGHNNGVCWHNQLFVTVVDTTRSTNLTICASTQSPVPGQYDATKFKQYSRHVEEYDLQFIFQLCTITLTADVMSYIHSMNSSILEDWNFGVPPPPTTSLVDTYRFVQSVAITCQKDAAPAENKDPYDKLKFWNVDLKEKFSLDLDQYPLGRKFLVQAGL

SEQ ID NO: 11 - protein, 528 aa, Artificial Sequence
  PEPTIDE (1)..(528): 18L1h4432-433/59dE
MALWRPSDNTVYLPPPSVARVVNTDDYVTRTSIFYHAGSSRLLTVGNPYFRVPAGGGNKQDIPKVSAYQYRVFRVQLPDPNKFGLPDTSIYNPETQRLVWACAGVEIGRGQPLGVGLSGHPFYNKLDDTESSHAATSNVSEDVRDNVSVDYKQTQLCILGCAPAIGEHWAKGTACKSRPLSQGDCPPLELKNTVLEDGDMVDTGYGAMDFSTLQDTKCEVPLDICQSICKYPDYLQMSADPYGDSMFFCLRREQLFARHFWNRAGTMGDTVPQSLYIKGTGMRASPGSCVYSPSPSGSIVTSDSQLFNKPYWLHKAQGHNNGVCWHNQLFVTVVDTTRSTNLTICASTQSPVPGQYDATKFKQYSRHVEEYDLQFIFQLCTITLTADVMSYIHSMNSSILEDWNFGVPPPPTTSLVDTYRFVQSVAITCQKDLYKTCKQAGTCPSDVINKVEGAAPAENKDPYDKLKFWNVDLKEKFSLDLDQYPLGRKFLVQAGLRRKPTIGPRKRSAPSATTSSKPAKRVRVRARK

SEQ ID NO: 12 - protein, 496 aa, Artificial Sequence
  PEPTIDE (1)..(496): 18L1 delta Ch4432-433/59dE
MALWRPSDNTVYLPPPSVARVVNTDDYVTRTSIFYHAGSSRLLTVGNPYFRVPAGGGNKQDIPKVSAYQYRVFRVQLPDPNKFGLPDTSIYNPETQRLVWACAGVEIGRGQPLGVGLSGHPFYNKLDDTESSHAATSNVSEDVRDNVSVDYKQTQLCILGCAPAIGEHWAKGTACKSRPLSQGDCPPLELKNTVLEDGDMVDTGYGAMDFSTLQDTKCEVPLDICQSICKYPDYLQMSADPYGDSMFFCLRREQLFARHFWNRAGTMGDTVPQSLYIKGTGMRASPGSCVYSPSPSGSIVTSDSQLFNKPYWLHKAQGHNNGVCWHNQLFVTVVDTTRSTNLTICASTQSPVPGQYDATKFKQYSRHVEEYDLQFIFQLCTITLTADVMSYIHSMNSSILEDWNFGVPPPPTTSLVDTYRFVQSVAITCQKDLYKTCKQAGTCPSDVINKVEGAAPAENKDPYDKLKFWNVDLKEKFSLDLDQYPLGRKFLVQAGL

SEQ ID NO: 13 - protein, 528 aa, Artificial Sequence
  PEPTIDE (1)..(528): 18L1h4434-435/59dE
MALWRPSDNTVYLPPPSVARVVNTDDYVTRTSIFYHAGSSRLLTVGNPYFRVPAGGGNKQDIPKVSAYQYRVFRVQLPDPNKFGLPDTSIYNPETQRLVWACAGVEIGRGQPLGVGLSGHPFYNKLDDTESSHAATSNVSEDVRDNVSVDYKQTQLCILGCAPAIGEHWAKGTACKSRPLSQGDCPPLELKNTVLEDGDMVDTGYGAMDFSTLQDTKCEVPLDICQSICKYPDYLQMSADPYGDSMFFCLRREQLFARHFWNRAGTMGDTVPQSLYIKGTGMRASPGSCVYSPSPSGSIVTSDSQLFNKPYWLHKAQGHNNGVCWHNQLFVTVVDTTRSTNLTICASTQSPVPGQYDATKFKQYSRHVEEYDLQFIFQLCTITLTADVMSYIHSMNSSILEDWNFGVPPPPTTSLVDTYRFVQSVAITCQKDAALYKTCKQAGTCPSDVINKVEGPAENKDPYDKLKFWNVDLKEKFSLDLDQYPLGRKFLVQAGLRRKPTIGPRKRSAPSATTSSKPAKRVRVRARK

SEQ ID NO: 14 - protein, 496 aa, Artificial Sequence
  PEPTIDE (1)..(496): 18L1 delta Ch4434-435/59dE
MALWRPSDNTVYLPPPSVARVVNTDDYVTRTSIFYHAGSSRLLTVGNPYFRVPAGGGNKQDIPKVSAYQYRVFRVQLPDPNKFGLPDTSIYNPETQRLVWACAGVEIGRGQPLGVGLSGHPFYNKLDDTESSHAATSNVSEDVRDNVSVDYKQTQLCILGCAPAIGEHWAKGTACKSRPLSQGDCPPLELKNTVLEDGDMVDTGYGAMDFSTLQDTKCEVPLDICQSICKYPDYLQMSADPYGDSMFFCLRREQLFARHFWNRAGTMGDTVPQSLYIKGTGMRASPGSCVYSPSPSGSIVTSDSQLFNKPYWLHKAQGHNNGVCWHNQLFVTVVDTTRSTNLTICASTQSPVPGQYDATKFKQYSRHVEEYDLQFIFQLCTITLTADVMSYIHSMNSSILEDWNFGVPPPPTTSLVDTYRFVQSVAITCQKDAALYKTCKQAGTCPSDVINKVEGPAENKDPYDKLKFWNVDLKEKFSLDLDQYPLGRKFLVQAGL

SEQ ID NO: 15 - protein, 526 aa, Artificial Sequence
  PEPTIDE (1)..(526): 18L1DE134-135/59dES
MALWRPSDNTVYLPPPSVARVVNTDDYVTRTSIFYHAGSSRLLTVGNPYFRVPAGGGNKQDIPKVSAYQYRVFRVQLPDPNKFGLPDTSIYNPETQRLVWACAGVEIGRGQPLGVGLSGHPFYNKLDDTESSHAGPLYKTCKQAGTCPSDVIPATSNVSEDVRDNVSVDYKQTQLCILGCAPAIGEHWAKGTACKSRPLSQGDCPPLELKNTVLEDGDMVDTGYGAMDFSTLQDTKCEVPLDICQSICKYPDYLQMSADPYGDSMFFCLRREQLFARHFWNRAGTMGDTVPQSLYIKGTGMRASPGSCVYSPSPSGSIVTSDSQLFNKPYWLHKAQGHNNGVCWHNQLFVTVVDTTRSTNLTICASTQSPVPGQYDATKFKQYSRHVEEYDLQFIFQLCTITLTADVMSYIHSMNSSILEDWNFGVPPPPTTSLVDTYRFVQSVAITCQKDAAPAENKDPYDKLKFWNVDLKEKFSLDLDQYPLGRKFLVQAGLRRKPTIGPRKRSAPSATTSSKPAKRVRVRARK

SEQ ID NO: 16 - protein, 494 aa, Artificial Sequence
  PEPTIDE (1)..(494): 18L1 delta CDE134-135/59dES
MALWRPSDNTVYLPPPSVARVVNTDDYVTRTSIFYHAGSSRLLTVGNPYFRVPAGGGNKQDIPKVSAYQYRVFRVQLPDPNKFGLPDTSIYNPETQRLVWACAGVEIGRGQPLGVGLSGHPFYNKLDDTESSHAGPLYKTCKQAGTCPSDVIPATSNVSEDVRDNVSVDYKQTQLCILGCAPAIGEHWAKGTACKSRPLSQGDCPPLELKNTVLEDGDMVDTGYGAMDFSTLQDTKCEVPLDICQSICKYPDYLQMSADPYGDSMFFCLRREQLFARHFWNRAGTMGDTVPQSLYIKGTGMRASPGSCVYSPSPSGSIVTSDSQLFNKPYWLHKAQGHNNGVCWHNQLFVTVVDTTRSTNLTICASTQSPVPGQYDATKFKQYSRHVEEYDLQFIFQLCTITLTADVMSYIHSMNSSILEDWNFGVPPPPTTSLVDTYRFVQSVAITCQKDAAPAENKDPYDKLKFWNVDLKEKFSLDLDQYPLGRKFLVQAGL

SEQ ID NO: 17 - protein, 532 aa, Artificial Sequence
  PEPTIDE (1)..(532): 18L1DE134-135/59dE
MALWRPSDNTVYLPPPSVARVVNTDDYVTRTSIFYHAGSSRLLTVGNPYFRVPAGGGNKQDIPKVSAYQYRVFRVQLPDPNKFGLPDTSIYNPETQRLVWACAGVEIGRGQPLGVGLSGHPFYNKLDDTESSHAGPDLYKTCKQAGTCPSDVINKVEGPATSNVSEDVRDNVSVDYKQTQLCILGCAPAIGEHWAKGTACKSRPLSQGDCPPLELKNTVLEDGDMVDTGYGAMDFSTLQDTKCEVPLDICQSICKYPDYLQMSADPYGDSMFFCLRREQLFARHFWNRAGTMGDTVPQSLYIKGTGMRASPGSCVYSPSPSGSIVTSDSQLFNKPYWLHKAQGHNNGVCWHNQLFVTVVDTTRSTNLTICASTQSPVPGQYDATKFKQYSRHVEEYDLQFIFQLCTITLTADVMSYIHSMNSSILEDWNFGVPPPPTTSLVDTYRFVQSVAITCQKDAAPAENKDPYDKLKFWNVDLKEKFSLDLDQYPLGRKFLVQAGLRRKPTIGPRKRSAPSATTSSKPAKRVRVRARK

SEQ ID NO: 18 - protein, 500 aa, Artificial Sequence
  PEPTIDE (1)..(500): 18L1 delta CDE134-135/59dE
MALWRPSDNTVYLPPPSVARVVNTDDYVTRTSIFYHAGSSRLLTVGNPYFRVPAGGGNKQDIPKVSAYQYRVFRVQLPDPNKFGLPDTSIYNPETQRLVWACAGVEIGRGQPLGVGLSGHPFYNKLDDTESSHAGPDLYKTCKQAGTCPSDVINKVEGPATSNVSEDVRDNVSVDYKQTQLCILGCAPAIGEHWAKGTACKSRPLSQGDCPPLELKNTVLEDGDMVDTGYGAMDFSTLQDTKCEVPLDICQSICKYPDYLQMSADPYGDSMFFCLRREQLFARHFWNRAGTMGDTVPQSLYIKGTGMRASPGSCVYSPSPSGSIVTSDSQLFNKPYWLHKAQGHNNGVCWHNQLFVTVVDTTRSTNLTICASTQSPVPGQYDATKFKQYSRHVEEYDLQFIFQLCTITLTADVMSYIHSMNSSILEDWNFGVPPPPTTSLVDTYRFVQSVAITCQKDAAPAENKDPYDKLKFWNVDLKEKFSLDLDQYPLGRKFLVQAGL

SEQ ID NO: 19 - protein, 524 aa, Artificial Sequence
  PEPTIDE (1)..(524): 18L1DE131-138/59dE
MALWRPSDNTVYLPPPSVARVVNTDDYVTRTSIFYHAGSSRLLTVGNPYFRVPAGGGNKQDIPKVSAYQYRVFRVQLPDPNKFGLPDTSIYNPETQRLVWACAGVEIGRGQPLGVGLSGHPFYNKLDDTESGPLYKTCKQAGTCPSDVINKVEGNVSEDVRDNVSVDYKQTQLCILGCAPAIGEHWAKGTACKSRPLSQGDCPPLELKNTVLEDGDMVDTGYGAMDFSTLQDTKCEVPLDICQSICKYPDYLQMSADPYGDSMFFCLRREQLFARHFWNRAGTMGDTVPQSLYIKGTGMRASPGSCVYSPSPSGSIVTSDSQLFNKPYWLHKAQGHNNGVCWHNQLFVTVVDTTRSTNLTICASTQSPVPGQYDATKFKQYSRHVEEYDLQFIFQLCTITLTADVMSYIHSMNSSILEDWNFGVPPPPTTSLVDTYRFVQSVAITCQKDAAPAENKDPYDKLKFWNVDLKEKFSLDLDQYPLGRKFLVQAGLRRKPTIGPRKRSAPSATTSSKPAKRVRVRARK

SEQ ID NO: 20 - protein, 492 aa, Artificial Sequence
  PEPTIDE (1)..(492): 18L1 delta CDE131-138/59dE
MALWRPSDNTVYLPPPSVARVVNTDDYVTRTSIFYHAGSSRLLTVGNPYFRVPAGGGNKQDIPKVSAYQYRVFRVQLPDPNKFGLPDTSIYNPETQRLVWACAGVEIGRGQPLGVGLSGHPFYNKLDDTESGPLYKTCKQAGTCPSDVINKVEGNVSEDVRDNVSVDYKQTQLCILGCAPAIGEHWAKGTACKSRPLSQGDCPPLELKNTVLEDGDMVDTGYGAMDFSTLQDTKCEVPLDICQSICKYPDYLQMSADPYGDSMFFCLRREQLFARHFWNRAGTMGDTVPQSLYIKGTGMRASPGSCVYSPSPSGSIVTSDSQLFNKPYWLHKAQGHNNGVCWHNQLFVTVVDTTRSTNLTICASTQSPVPGQYDATKFKQYSRHVEEYDLQFIFQLCTITLTADVMSYIHSMNSSILEDWNFGVPPPPTTSLVDTYRFVQSVAITCQKDAAPAENKDPYDKLKFWNVDLKEKFSLDLDQYPLGRKFLVQAGL

SEQ ID NO: 21 - protein, 526 aa, Artificial Sequence
  PEPTIDE (1)..(526): 18L1DE121-124/59dE
MALWRPSDNTVYLPPPSVARVVNTDDYVTRTSIFYHAGSSRLLTVGNPYFRVPAGGGNKQDIPKVSAYQYRVFRVQLPDPNKFGLPDTSIYNPETQRLVWACAGVEIGRGQPLGVGLSGHPLYKTCKQAGTCPSDVINKVEGNKLDDTESSHAATSNVSEDVRDNVSVDYKQTQLCILGCAPAIGEHWAKGTACKSRPLSQGDCPPLELKNTVLEDGDMVDTGYGAMDFSTLQDTKCEVPLDICQSICKYPDYLQMSADPYGDSMFFCLRREQLFARHFWNRAGTMGDTVPQSLYIKGTGMRASPGSCVYSPSPSGSIVTSDSQLFNKPYWLHKAQGHNNGVCWHNQLFVTVVDTTRSTNLTICASTQSPVPGQYDATKFKQYSRHVEEYDLQFIFQLCTITLTADVMSYIHSMNSSILEDWNFGVPPPPTTSLVDTYRFVQSVAITCQKDAAPAENKDPYDKLKFWNVDLKEKFSLDLDQYPLGRKFLVQAGLRRKPTIGPRKRSAPSATTSSKPAKRVRVRARK

SEQ ID NO: 22 - protein, 494 aa, Artificial Sequence
  PEPTIDE (1)..(494): 18L1 delta CDE121-124/59dE
MALWRPSDNTVYLPPPSVARVVNTDDYVTRTSIFYHAGSSRLLTVGNPYFRVPAGGGNKQDIPKVSAYQYRVFRVQLPDPNKFGLPDTSIYNPETQRLVWACAGVEIGRGQPLGVGLSGHPLYKTCKQAGTCPSDVINKVEGNKLDDTESSHAATSNVSEDVRDNVSVDYKQTQLCILGCAPAIGEHWAKGTACKSRPLSQGDCPPLELKNTVLEDGDMVDTGYGAMDFSTLQDTKCEVPLDICQSICKYPDYLQMSADPYGDSMFFCLRREQLFARHFWNRAGTMGDTVPQSLYIKGTGMRASPGSCVYSPSPSGSIVTSDSQLFNKPYWLHKAQGHNNGVCWHNQLFVTVVDTTRSTNLTICASTQSPVPGQYDATKFKQYSRHVEEYDLQFIFQLCTITLTADVMSYIHSMNSSILEDWNFGVPPPPTTSLVDTYRFVQSVAITCQKDAAPAENKDPYDKLKFWNVDLKEKFSLDLDQYPLGRKFLVQAGL

SEQ ID NO: 23 - protein, 527 aa, Artificial Sequence
  PEPTIDE (1)..(527): 18L1h4431-433/59dE
MALWRPSDNTVYLPPPSVARVVNTDDYVTRTSIFYHAGSSRLLTVGNPYFRVPAGGGNKQDIPKVSAYQYRVFRVQLPDPNKFGLPDTSIYNPETQRLVWACAGVEIGRGQPLGVGLSGHPFYNKLDDTESSHAATSNVSEDVRDNVSVDYKQTQLCILGCAPAIGEHWAKGTACKSRPLSQGDCPPLELKNTVLEDGDMVDTGYGAMDFSTLQDTKCEVPLDICQSICKYPDYLQMSADPYGDSMFFCLRREQLFARHFWNRAGTMGDTVPQSLYIKGTGMRASPGSCVYSPSPSGSIVTSDSQLFNKPYWLHKAQGHNNGVCWHNQLFVTVVDTTRSTNLTICASTQSPVPGQYDATKFKQYSRHVEEYDLQFIFQLCTITLTADVMSYIHSMNSSILEDWNFGVPPPPTTSLVDTYRFVQSVAITCQKLYKTCKQAGTCPSDVINKVEGAAPAENKDPYDKLKFWNVDLKEKFSLDLDQYPLGRKFLVQAGLRRKPTIGPRKRSAPSATTSSKPAKRVRVRARK

SEQ ID NO: 24 - protein, 495 aa, Artificial Sequence
  PEPTIDE (1)..(495): 18L1 delta Ch4431-433/59dE
MALWRPSDNTVYLPPPSVARVVNTDDYVTRTSIFYHAGSSRLLTVGNPYFRVPAGGGNKQDIPKVSAYQYRVFRVQLPDPNKFGLPDTSIYNPETQRLVWACAGVEIGRGQPLGVGLSGHPFYNKLDDTESSHAATSNVSEDVRDNVSVDYKQTQLCILGCAPAIGEHWAKGTACKSRPLSQGDCPPLELKNTVLEDGDMVDTGYGAMDFSTLQDTKCEVPLDICQSICKYPDYLQMSADPYGDSMFFCLRREQLFARHFWNRAGTMGDTVPQSLYIKGTGMRASPGSCVYSPSPSGSIVTSDSQLFNKPYWLHKAQGHNNGVCWHNQLFVTVVDTTRSTNLTICASTQSPVPGQYDATKFKQYSRHVEEYDLQFIFQLCTITLTADVMSYIHSMNSSILEDWNFGVPPPPTTSLVDTYRFVQSVAITCQKLYKTCKQAGTCPSDVINKVEGAAPAENKDPYDKLKFWNVDLKEKFSLDLDQYPLGRKFLVQAGL

SEQ ID NO: 25 - protein, 526 aa, Artificial Sequence
  PEPTIDE (1)..(526): 18L1h4432-435/59dE
MALWRPSDNTVYLPPPSVARVVNTDDYVTRTSIFYHAGSSRLLTVGNPYFRVPAGGGNKQDIPKVSAYQYRVFRVQLPDPNKFGLPDTSIYNPETQRLVWACAGVEIGRGQPLGVGLSGHPFYNKLDDTESSHAATSNVSEDVRDNVSVDYKQTQLCILGCAPAIGEHWAKGTACKSRPLSQGDCPPLELKNTVLEDGDMVDTGYGAMDFSTLQDTKCEVPLDICQSICKYPDYLQMSADPYGDSMFFCLRREQLFARHFWNRAGTMGDTVPQSLYIKGTGMRASPGSCVYSPSPSGSIVTSDSQLFNKPYWLHKAQGHNNGVCWHNQLFVTVVDTTRSTNLTICASTQSPVPGQYDATKFKQYSRHVEEYDLQFIFQLCTITLTADVMSYIHSMNSSILEDWNFGVPPPPTTSLVDTYRFVQSVAITCQKDLYKTCKQAGTCPSDVINKVEGPAENKDPYDKLKFWNVDLKEKFSLDLDQYPLGRKFLVQAGLRRKPTIGPRKRSAPSATTSSKPAKRVRVRARK

SEQ ID NO: 26 - protein, 494 aa, Artificial Sequence
  PEPTIDE (1)..(494): 18L1 delta Ch4432-435/59dE
MALWRPSDNTVYLPPPSVARVVNTDDYVTRTSIFYHAGSSRLLTVGNPYFRVPAGGGNKQDIPKVSAYQYRVFRVQLPDPNKFGLPDTSIYNPETQRLVWACAGVEIGRGQPLGVGLSGHPFYNKLDDTESSHAATSNVSEDVRDNVSVDYKQTQLCILGCAPAIGEHWAKGTACKSRPLSQGDCPPLELKNTVLEDGDMVDTGYGAMDFSTLQDTKCEVPLDICQSICKYPDYLQMSADPYGDSMFFCLRREQLFARHFWNRAGTMGDTVPQSLYIKGTGMRASPGSCVYSPSPSGSIVTSDSQLFNKPYWLHKAQGHNNGVCWHNQLFVTVVDTTRSTNLTICASTQSPVPGQYDATKFKQYSRHVEEYDLQFIFQLCTITLTADVMSYIHSMNSSILEDWNFGVPPPPTTSLVDTYRFVQSVAITCQKDLYKTCKQAGTCPSDVINKVEGPAENKDPYDKLKFWNVDLKEKFSLDLDQYPLGRKFLVQAGL

SEQ ID NO: 27 - protein, 523 aa, Artificial Sequence
  PEPTIDE (1)..(523): 18L1DE137-138/59dES-mut1
MALWRPSDNTVYLPPPSVARVVNTDDYVTRTSIFYHAGSSRLLTVGNPYFRVPAGGGNKQDIPKVSAYQYRVFRVQLPDPNKFGLPDTSIYNPETQRLVWACAGVEIGRGQPLGVGLSGHPFYNKLDDTESSHAATSLYKTCKQAGTCPSDVINVSEDVRDNVSVDYKQTQLCILGCAPAIGEHWAKGTACKSRPLSQGDCPPLELKNTVLEDGDMVDTGYGAMDFSTLQDTKCEVPLDICQSICKYPDYLQMSADPYGDSMFFCLRREQLFARHFWNRAGTMGDTVPQSLYIKGTGMRASPGSCVYSPSPSGSIVTSDSQLFNKPYWLHKAQGHNNGVCWHNQLFVTVVDTTRSTNLTICASTQSPVPGQYDATKFKQYSRHVEEYDLQFIFQLCTITLTADVMSYIHSMNSSILEDWNFGVPPPPTTSLVDTYRFVQSVAITCQKDAAPAENKDPYDKLKFWNVDLKEKFSLDLDQYPLGRKFLVQAGLRGGPTIGPGSRSAPSATTSSGPAGSVSVGAGK

SEQ ID NO: 28 - protein, 523 aa, Artificial Sequence
  PEPTIDE (1)..(523): 18L1DE137-138/59dES-mut2
MALWRPSDNTVYLPPPSVARVVNTDDYVTRTSIFYHAGSSRLLTVGNPYFRVPAGGGNKQDIPKVSAYQYRVFRVQLPDPNKFGLPDTSIYNPETQRLVWACAGVEIGRGQPLGVGLSGHPFYNKLDDTESSHAATSLYKTCKQAGTCPSDVINVSEDVRDNVSVDYKQTQLCILGCAPAIGEHWAKGTACKSRPLSQGDCPPLELKNTVLEDGDMVDTGYGAMDFSTLQDTKCEVPLDICQSICKYPDYLQMSADPYGDSMFFCLRREQLFARHFWNRAGTMGDTVPQSLYIKGTGMRASPGSCVYSPSPSGSIVTSDSQLFNKPYWLHKAQGHNNGVCWHNQLFVTVVDTTRSTNLTICASTQSPVPGQYDATKFKQYSRHVEEYDLQFIFQLCTITLTADVMSYIHSMNSSILEDWNFGVPPPPTTSLVDTYRFVQSVAITCQKDAAPAENKDPYDKLKFWNVDLKEKFSLDLDQYPLGRKFLVQAGLRGGPTIGPRGSSAPSATTSSGPAGSVSVGAGK

SEQ ID NO: 29 - protein, 523 aa, Artificial Sequence
  PEPTIDE (1)..(523): 18L1DE137-138/59dES-mut3
MALWRPSDNTVYLPPPSVARVVNTDDYVTRTSIFYHAGSSRLLTVGNPYFRVPAGGGNKQDIPKVSAYQYRVFRVQLPDPNKFGLPDTSIYNPETQRLVWACAGVEIGRGQPLGVGLSGHPFYNKLDDTESSHAATSLYKTCKQAGTCPSDVINVSEDVRDNVSVDYKQTQLCILGCAPAIGEHWAKGTACKSRPLSQGDCPPLELKNTVLEDGDMVDTGYGAMDFSTLQDTKCEVPLDICQSICKYPDYLQMSADPYGDSMFFCLRREQLFARHFWNRAGTMGDTVPQSLYIKGTGMRASPGSCVYSPSPSGSIVTSDSQLFNKPYWLHKAQGHNNGVCWHNQLFVTVVDTTRSTNLTICASTQSPVPGQYDATKFKQYSRHVEEYDLQFIFQLCTITLTADVMSYIHSMNSSILEDWNFGVPPPPTTSLVDTYRFVQSVAITCQKDAAPAENKDPYDKLKFWNVDLKEKFSLDLDQYPLGRKFLVQAGLRGGPTIGPGSRSAPSATTSSGPAGSVGVDAGK

SEQ ID NO: 30 - protein, 523 aa, Artificial Sequence
  PEPTIDE (1)..(523): 18L1DE137-138/59dES-mut4
MALWRPSDNTVYLPPPSVARVVNTDDYVTRTSIFYHAGSSRLLTVGNPYFRVPAGGGNKQDIPKVSAYQYRVFRVQLPDPNKFGLPDTSIYNPETQRLVWACAGVEIGRGQPLGVGLSGHPFYNKLDDTESSHAATSLYKTCKQAGTCPSDVINVSEDVRDNVSVDYKQTQLCILGCAPAIGEHWAKGTACKSRPLSQGDCPPLELKNTVLEDGDMVDTGYGAMDFSTLQDTKCEVPLDICQSICKYPDYLQMSADPYGDSMFFCLRREQLFARHFWNRAGTMGDTVPQSLYIKGTGMRASPGSCVYSPSPSGSIVTSDSQLFNKPYWLHKAQGHNNGVCWHNQLFVTVVDTTRSTNLTICASTQSPVPGQYDATKFKQYSRHVEEYDLQFIFQLCTITLTADVMSYIHSMNSSILEDWNFGVPPPPTTSLVDTYRFVQSVAITCQKDAAPAENKDPYDKLKFWNVDLKEKFSLDLDQYPLGRKFLVQAGLRGGPTIGPRGSSAPSATTSSGPADSVGVDAGK

SEQ ID NO: 31 - protein, 523 aa, Artificial Sequence
  PEPTIDE (1)..(523): 18L1DE137-138/59dES-mut5
MALWRPSDNTVYLPPPSVARVVNTDDYVTRTSIFYHAGSSRLLTVGNPYFRVPAGGGNKQDIPKVSAYQYRVFRVQLPDPNKFGLPDTSIYNPETQRLVWACAGVEIGRGQPLGVGLSGHPFYNKLDDTESSHAATSLYKTCKQAGTCPSDVINVSEDVRDNVSVDYKQTQLCILGCAPAIGEHWAKGTACKSRPLSQGDCPPLELKNTVLEDGDMVDTGYGAMDFSTLQDTKCEVPLDICQSICKYPDYLQMSADPYGDSMFFCLRREQLFARHFWNRAGTMGDTVPQSLYIKGTGMRASPGSCVYSPSPSGSIVTSDSQLFNKPYWLHKAQGHNNGVCWHNQLFVTVVDTTRSTNLTICASTQSPVPGQYDATKFKQYSRHVEEYDLQFIFQLCTITLTADVMSYIHSMNSSILEDWNFGVPPPPTTSLVDTYRFVQSVAITCQKDAAPAENKDPYDKLKFWNVDLKEKFSLDLDQYPLGRKFLVQAGLRGKPTIGPGSRSAPSATTSSGPAGSVSVGAGK

SEQ ID NO: 32 - protein, 523 aa, Artificial Sequence
  PEPTIDE (1)..(523): 18L1DE137-138/59dES-mut6
MALWRPSDNTVYLPPPSVARVVNTDDYVTRTSIFYHAGSSRLLTVGNPYFRVPAGGGNKQDIPKVSAYQYRVFRVQLPDPNKFGLPDTSIYNPETQRLVWACAGVEIGRGQPLGVGLSGHPFYNKLDDTESSHAATSLYKTCKQAGTCPSDVINVSEDVRDNVSVDYKQTQLCILGCAPAIGEHWAKGTACKSRPLSQGDCPPLELKNTVLEDGDMVDTGYGAMDFSTLQDTKCEVPLDICQSICKYPDYLQMSADPYGDSMFFCLRREQLFARHFWNRAGTMGDTVPQSLYIKGTGMRASPGSCVYSPSPSGSIVTSDSQLFNKPYWLHKAQGHNNGVCWHNQLFVTVVDTTRSTNLTICASTQSPVPGQYDATKFKQYSRHVEEYDLQFIFQLCTITLTADVMSYIHSMNSSILEDWNFGVPPPPTTSLVDTYRFVQSVAITCQKDAAPAENKDPYDKLKFWNVDLKEKFSLDLDQYPLGRKFLVQAGLRGKPTIGPRGSSAPSATTSSGPAGSVSVGAGK

SEQ ID NO: 33 - DNA, 1477 bp, Artificial Sequence
  EXON (1)..(1477): 18L1 delta CDE137-138/59dES nt
atggctctctggagaccctccgataacacagtgtacttgcccccccccagcgtcgcccgcgtcgtgaacacagacgactacgtcaccaggacctcaatcttctaccacgccggttcaagccgcctgctgaccgtcggcaacccctacttccgcgtccccgccggtggcggtaacaaacaagacatccccaaagtcagcgcctatcagtaccgcgtgttccgcgtccaactgcccgatcccaacaagttcggcctgcccgacacctccatctacaaccccgagacccagaggctggtctgggcatgcgccggcgtcgagatcggtaggggccaacccctgggcgtcggtttgtccggccaccccttctacaacaagctggacgataccgagtcctcccacgcagcaaccagcctgtacaagacctgcaagcaggccggtacctgcccctccgacgtcatcaacgtcagcgaagatgtccgcgataacgtcagcgtggactacaaacaaacccaactgtgcatcctcggttgcgcacccgccatcggcgagcattgggccaagggtaccgcctgcaagagcaggcccctgagccaaggtgactgtccacccctggagttgaagaataccgtcctcgaggacggcgacatggtggacaccggctacggcgcaatggatttctccaccctgcaggacaccaagtgcgaagtgcccctcgacatctgccaaagcatctgcaagtaccccgactacctgcagatgagcgccgacccctacggcgactccatgttcttctgtctgagaagggaacaattgttcgcccgccacttctggaaccgcgccggcaccatgggcgataccgtcccccagtccctgtacatcaagggtaccggcatgagggccagccccggttcatgcgtctacagcccaagcccctccggtagcatcgtcacaagcgattcccaactcttcaacaagccctactggctgcacaaagcccaaggccacaataacggcgtctgttggcacaaccagctgttcgtcaccgtcgtggacacaaccaggtccacaaacctgaccatctgcgccagcacccaaagccccgtgcccggccagtacgacgccacaaagttcaaacaatactcacgccacgtcgaagagtacgacctccaattcatcttccaactctgcaccatcaccctgaccgccgacgtcatgtcctacatccactccatgaactcatccatcctggaagactggaatttcggcgtcccaccaccccccaccacctccctcgtcgacacctacaggttcgtgcagagcgtcgccatcacatgccagaaagacgccgcccccgccgagaacaaagacccatacgacaaactgaaattctggaacgtcgacctgaaagagaaattcagcctggatctggaccagtacccattgggcaggaagttcctcgtccaggcgggtctctaat

SEQ ID NO: 34 - DNA, 1489 bp, Artificial Sequence
  EXON (1)..(1489): 18L1 delta CDE137-138/59dE nt
atggctctctggagaccctccgataacacagtgtacttgcccccccccagcgtcgcccgcgtcgtgaacacagacgactacgtcaccaggacctcaatcttctaccacgccggttcaagccgcctgctgaccgtcggcaacccctacttccgcgtccccgccggtggcggtaacaaacaagacatccccaaagtcagcgcctatcagtaccgcgtgttccgcgtccaactgcccgatcccaacaagttcggcctgcccgacacctccatctacaaccccgagacccagaggctggtctgggcatgcgccggcgtcgagatcggtaggggccaacccctgggcgtcggtttgtccggccaccccttctacaacaagctggacgataccgagtcctcccacgcagcaaccagcgacctgtacaagacctgcaagcaggccggtacctgcccctccgacgtcatcaacaaggtcaacgtcagcgaagatgtccgcgataacgtcagcgtggactacaaacaaacccaactgtgcatcctcggttgcgcacccgccatcggcgagcattgggccaagggtaccgcctgcaagagcaggcccctgagccaaggtgactgtccacccctggagttgaagaataccgtcctcgaggacggcgacatggtggacaccggctacggcgcaatggatttctccaccctgcaggacaccaagtgcgaagtgcccctcgacatctgccaaagcatctgcaagtaccccgactacctgcagatgagcgccgacccctacggcgactccatgttcttctgtctgagaagggaacaattgttcgcccgccacttctggaaccgcgccggcaccatgggcgataccgtcccccagtccctgtacatcaagggtaccggcatgagggccagccccggttcatgcgtctacagcccaagcccctccggtagcatcgtcacaagcgattcccaactcttcaacaagccctactggctgcacaaagcccaaggccacaataacggcgtctgttggcacaaccagctgttcgtcaccgtcgtggacacaaccaggtccacaaacctgaccatctgcgccagcacccaaagccccgtgcccggccagtacgacgccacaaagttcaaacaatactcacgccacgtcgaagagtacgacctccaattcatcttccaactctgcaccatcaccctgaccgccgacgtcatgtcctacatccactccatgaactcatccatcctggaagactggaatttcggcgtcccaccaccccccaccacctccctcgtcgacacctacaggttcgtgcagagcgtcgccatcacatgccagaaagacgccgcccccgccgagaacaaagacccatacgacaaactgaaattctggaacgtcgacctgaaagagaaattcagcctggatctggaccagtacccattgggcaggaagttcctcgtccaggcgggtctctaat

SEQ ID NO: 35 - DNA, 1486 bp, Artificial Sequence
  EXON (1)..(1486): 18L1 delta CDE134-135/59dES nt
atggctctctggagaccctccgataacacagtgtacttgcccccccccagcgtcgcccgcgtcgtgaacacagacgactacgtcaccaggacctcaatcttctaccacgccggttcaagccgcctgctgaccgtcggcaacccctacttccgcgtccccgccggtggcggtaacaaacaagacatccccaaagtcagcgcctatcagtaccgcgtgttccgcgtccaactgcccgatcccaacaagttcggcctgcccgacacctccatctacaaccccgagacccagaggctggtctgggcatgcgccggcgtcgagatcggtaggggccaacccctgggcgtcggtttgtccggccaccccttctacaacaagctggacgataccgagtcctcccacgcaggaccactgtacaagacctgcaagcaggccggtacctgcccctccgacgtcatcccagcaaccagcaacgtcagcgaagatgtccgcgataacgtcagcgtggactacaaacaaacccaactgtgcatcctcggttgcgcacccgccatcggcgagcattgggccaagggtaccgcctgcaagagcaggcccctgagccaaggtgactgtccacccctggagttgaagaataccgtcctcgaggacggcgacatggtggacaccggctacggcgcaatggatttctccaccctgcaggacaccaagtgcgaagtgcccctcgacatctgccaaagcatctgcaagtaccccgactacctgcagatgagcgccgacccctacggcgactccatgttcttctgtctgagaagggaacaattgttcgcccgccacttctggaaccgcgccggcaccatgggcgataccgtcccccagtccctgtacatcaagggtaccggcatgagggccagccccggttcatgcgtctacagcccaagcccctccggtagcatcgtcacaagcgattcccaactcttcaacaagccctactggctgcacaaagcccaaggccacaataacggcgtctgttggcacaaccagctgttcgtcaccgtcgtggacacaaccaggtccacaaacctgaccatctgcgccagcacccaaagccccgtgcccggccagtacgacgccacaaagttcaaacaatactcacgccacgtcgaagagtacgacctccaattcatcttccaactctgcaccatcaccctgaccgccgacgtcatgtcctacatccactccatgaactcatccatcctggaagactggaatttcggcgtcccaccaccccccaccacctccctcgtcgacacctacaggttcgtgcagagcgtcgccatcacatgccagaaagacgccgcccccgccgagaacaaagacccatacgacaaactgaaattctggaacgtcgacctgaaagagaaattcagcctggatctggaccagtacccattgggcaggaagttcctcgtccaggcgggtctctaat

SEQ ID NO: 36 - DNA, 1504 bp, Artificial Sequence
  EXON (1)..(1504): 18L1 delta CDE134-135/59dE nt
atggctctctggagaccctccgataacacagtgtacttgcccccccccagcgtcgcccgcgtcgtgaacacagacgactacgtcaccaggacctcaatcttctaccacgccggttcaagccgcctgctgaccgtcggcaacccctacttccgcgtccccgccggtggcggtaacaaacaagacatccccaaagtcagcgcctatcagtaccgcgtgttccgcgtccaactgcccgatcccaacaagttcggcctgcccgacacctccatctacaaccccgagacccagaggctggtctgggcatgcgccggcgtcgagatcggtaggggccaacccctgggcgtcggtttgtccggccaccccttctacaacaagctggacgataccgagtcctcccacgcaggaccagacctgtacaagacctgcaagcaggccggtacctgcccctccgacgtcatcaacaaggtcgaaggaccagcaaccagcaacgtcagcgaagatgtccgcgataacgtcagcgtggactacaaacaaacccaactgtgcatcctcggttgcgcacccgccatcggcgagcattgggccaagggtaccgcctgcaagagcaggcccctgagccaaggtgactgtccacccctggagttgaagaataccgtcctcgaggacggcgacatggtggacaccggctacggcgcaatggatttctccaccctgcaggacaccaagtgcgaagtgcccctcgacatctgccaaagcatctgcaagtaccccgactacctgcagatgagcgccgacccctacggcgactccatgttcttctgtctgagaagggaacaattgttcgcccgccacttctggaaccgcgccggcaccatgggcgataccgtcccccagtccctgtacatcaagggtaccggcatgagggccagccccggttcatgcgtctacagcccaagcccctccggtagcatcgtcacaagcgattcccaactcttcaacaagccctactggctgcacaaagcccaaggccacaataacggcgtctgttggcacaaccagctgttcgtcaccgtcgtggacacaaccaggtccacaaacctgaccatctgcgccagcacccaaagccccgtgcccggccagtacgacgccacaaagttcaaacaatactcacgccacgtcgaagagtacgacctccaattcatcttccaactctgcaccatcaccctgaccgccgacgtcatgtcctacatccactccatgaactcatccatcctggaagactggaatttcggtgtcccaccaccccccaccacctccctcgtcgacacctacaggttcgtgcagagcgtcgccatcacatgccagaaagacgccgcccccgccgagaacaaagacccatacgacaaactgaaattctggaacgtcgacctgaaagagaaattcagcctggatctggaccagtacccattgggcaggaagttcctcgtccaggcgggtctctaat

SEQ ID NO: 37 - DNA, 1480 bp, Artificial Sequence
  EXON (1)..(1480): 18L1 delta CDE131-138/59dE nt
atggctctctggagaccctccgataacacagtgtacttgcccccccccagcgtcgcccgcgtcgtgaacacagacgactacgtcaccaggacctcaatcttctaccacgccggttcaagccgcctgctgaccgtcggcaacccctacttccgcgtccccgccggtggcggtaacaaacaagacatccccaaagtcagcgcctatcagtaccgcgtgttccgcgtccaactgcccgatcccaacaagttcggcctgcccgacacctccatctacaaccccgagacccagaggctggtctgggcatgcgccggcgtcgagatcggtaggggccaacccctgggcgtcggtttgtccggccaccccttctacaacaagctggacgataccgagtccggtcccctgtacaagacctgcaagcaggccggtacctgcccctccgacgtcatcaacaaggtcgaaggaaacgtcagcgaagatgtccgcgataacgtcagcgtggactacaaacaaacccaactgtgcatcctcggttgcgcacccgccatcggcgagcattgggccaagggtaccgcctgcaagagcaggcccctgagccaaggtgactgtccacccctggagttgaagaataccgtcctcgaggacggcgacatggtggacaccggctacggcgcaatggatttctccaccctgcaggacaccaagtgcgaagtgcccctcgacatctgccaaagcatctgcaagtaccccgactacctgcagatgagcgccgacccctacggcgactccatgttcttctgtctgagaagggaacaattgttcgcccgccacttctggaaccgcgccggcaccatgggcgataccgtcccccagtccctgtacatcaagggtaccggcatgagggccagccccggttcatgcgtctacagcccaagcccctccggtagcatcgtcacaagcgattcccaactcttcaacaagccctactggctgcacaaagcccaaggccacaataacggcgtctgttggcacaaccagctgttcgtcaccgtcgtggacacaaccaggtccacaaacctgaccatctgcgccagcacccaaagccccgtgcccggccagtacgacgccacaaagttcaaacaatactcacgccacgtcgaagagtacgacctccaattcatcttccaactctgcaccatcaccctgaccgccgacgtcatgtcctacatccactccatgaactcatccatcctggaagactggaatttcggcgtcccaccaccccccaccacctccctcgtcgacacctacaggttcgtgcagagcgtcgccatcacatgccagaaagacgccgcccccgccgagaacaaagacccatacgacaaactgaaattctggaacgtcgacctgaaagagaaattcagcctggatctggaccagtacccattgggcaggaagttcctcgtccaggcgggtctctaat

SEQ ID NO: 38 - DNA, 1573 bp, Artificial Sequence
  EXON (1)..(1573): 18L1DE137-138/59dES-mut1 nt
atggctctctggagaccctccgataacacagtgtacttgcccccccccagcgtcgcccgcgtcgtgaacacagacgactacgtcaccaggacctcaatcttctaccacgccggttcaagccgcctgctgaccgtcggcaacccctacttccgcgtccccgccggtggcggtaacaaacaagacatccccaaagtcagcgcctatcagtaccgcgtgttccgcgtccaactgcccgatcccaacaagttcggcctgcccgacacctccatctacaaccccgagacccagaggctggtctgggcatgcgccggcgtcgagatcggtaggggccaacccctgggcgtcggtttgtccggccaccccttctacaacaagctggacgataccgagtcctcccacgcagcaaccagcctgtacaagacctgcaagcaggccggtacctgcccctccgacgtcatcaacgtcagcgaagatgtccgcgataacgtcagcgtggactacaaacaaacccaactgtgcatcctcggttgcgcacccgccatcggcgagcattgggccaagggtaccgcctgcaagagcaggcccctgagccaaggtgactgtccacccctggagttgaagaataccgtcctcgaggacggcgacatggtggacaccggctacggcgcaatggatttctccaccctgcaggacaccaagtgcgaagtgcccctcgacatctgccaaagcatctgcaagtaccccgactacctgcagatgagcgccgacccctacggcgactccatgttcttctgtctgagaagggaacaattgttcgcccgccacttctggaaccgcgccggcaccatgggcgataccgtcccccagtccctgtacatcaagggtaccggcatgagggccagccccggttcatgcgtctacagcccaagcccctccggtagcatcgtcacaagcgattcccaactcttcaacaagccctactggctgcacaaagcccaaggccacaataacggcgtctgttggcacaaccagctgttcgtcaccgtcgtggacacaaccaggtccacaaacctgaccatctgcgccagcacccaaagccccgtgcccggccagtacgacgccacaaagttcaaacaatactcacgccacgtcgaagagtacgacctccaattcatcttccaactctgcaccatcaccctgaccgccgacgtcatgtcctacatccactccatgaactcatccatcctggaagactggaatttcggcgtcccaccaccccccaccacctccctcgtcgacacctacaggttcgtgcagagcgtcgccatcacatgccagaaagacgccgcccccgccgagaacaaagacccatacgacaaactgaaattctggaacgtcgacctgaaagagaaattcagcctggatctggaccagtacccattgggcaggaagttcctcgtccaggcgggtctccgtggcggtccgacgattggccctggctctcgttctgccccgtcggccacgaccagcagcggccctgccggtagcgtgagcgtgggcgctggcaaataat

SEQ ID NO: 39 - DNA, 1573 bp, Artificial Sequence
  EXON (1)..(1573): 18L1DE137-138/59dES-mut2 nt
atggctctctggagaccctccgataacacagtgtacttgcccccccccagcgtcgcccgcgtcgtgaacacagacgactacgtcaccaggacctcaatcttctaccacgccggttcaagccgcctgctgaccgtcggcaacccctacttccgcgtccccgccggtggcggtaacaaacaagacatccccaaagtcagcgcctatcagtaccgcgtgttccgcgtccaactgcccgatcccaacaagttcggcctgcccgacacctccatctacaaccccgagacccagaggctggtctgggcatgcgccggcgtcgagatcggtaggggccaacccctgggcgtcggtttgtccggccaccccttctacaacaagctggacgataccgagtcctcccacgcagcaaccagcctgtacaagacctgcaagcaggccggtacctgcccctccgacgtcatcaacgtcagcgaagatgtccgcgataacgtcagcgtggactacaaacaaacccaactgtgcatcctcggttgcgcacccgccatcggcgagcattgggccaagggtaccgcctgcaagagcaggcccctgagccaaggtgactgtccacccctggagttgaagaataccgtcctcgaggacggcgacatggtggacaccggctacggcgcaatggatttctccaccctgcaggacaccaagtgcgaagtgcccctcgacatctgccaaagcatctgcaagtaccccgactacctgcagatgagcgccgacccctacggcgactccatgttcttctgtctgagaagggaacaattgttcgcccgccacttctggaaccgcgccggcaccatgggcgataccgtcccccagtccctgtacatcaagggtaccggcatgagggccagccccggttcatgcgtctacagcccaagcccctccggtagcatcgtcacaagcgattcccaactcttcaacaagccctactggctgcacaaagcccaaggccacaataacggcgtctgttggcacaaccagctgttcgtcaccgtcgtggacacaaccaggtccacaaacctgaccatctgcgccagcacccaaagccccgtgcccggccagtacgacgccacaaagttcaaacaatactcacgccacgtcgaagagtacgacctccaattcatcttccaactctgcaccatcaccctgaccgccgacgtcatgtcctacatccactccatgaactcatccatcctggaagactggaatttcggcgtcccaccaccccccaccacctccctcgtcgacacctacaggttcgtgcagagcgtcgccatcacatgccagaaagacgccgcccccgccgagaacaaagacccatacgacaaactgaaattctggaacgtcgacctgaaagagaaattcagcctggatctggaccagtacccattgggcaggaagttcctcgtccaggcgggtctccgtggcggtccgacgattggccctcgtggctcttctgccccgtcggccacgaccagcagcggccctgccggtagcgtgagcgtgggcgctggcaaataat

SEQ ID NO: 40 - DNA, 1573 bp, Artificial Sequence
  EXON (1)..(1573): 18L1DE137-138/59dES-mut3 nt
atggctctctggagaccctccgataacacagtgtacttgcccccccccagcgtcgcccgcgtcgtgaacacagacgactacgtcaccaggacctcaatcttctaccacgccggttcaagccgcctgctgaccgtcggcaacccctacttccgcgtccccgccggtggcggtaacaaacaagacatccccaaagtcagcgcctatcagtaccgcgtgttccgcgtccaactgcccgatcccaacaagttcggcctgcccgacacctccatctacaaccccgagacccagaggctggtctgggcatgcgccggcgtcgagatcggtaggggccaacccctgggcgtcggtttgtccggccaccccttctacaacaagctggacgataccgagtcctcccacgcagcaaccagcctgtacaagacctgcaagcaggccggtacctgcccctccgacgtcatcaacgtcagcgaagatgtccgcgataacgtcagcgtggactacaaacaaacccaactgtgcatcctcggttgcgcacccgccatcggcgagcattgggccaagggtaccgcctgcaagagcaggcccctgagccaaggtgactgtccacccctggagttgaagaataccgtcctcgaggacggcgacatggtggacaccggctacggcgcaatggatttctccaccctgcaggacaccaagtgcgaagtgcccctcgacatctgccaaagcatctgcaagtaccccgactacctgcagatgagcgccgacccctacggcgactccatgttcttctgtctgagaagggaacaattgttcgcccgccacttctggaaccgcgccggcaccatgggcgataccgtcccccagtccctgtacatcaagggtaccggcatgagggccagccccggttcatgcgtctacagcccaagcccctccggtagcatcgtcacaagcgattcccaactcttcaacaagccctactggctgcacaaagcccaaggccacaataacggcgtctgttggcacaaccagctgttcgtcaccgtcgtggacacaaccaggtccacaaacctgaccatctgcgccagcacccaaagccccgtgcccggccagtacgacgccacaaagttcaaacaatactcacgccacgtcgaagagtacgacctccaattcatcttccaactctgcaccatcaccctgaccgccgacgtcatgtcctacatccactccatgaactcatccatcctggaagactggaatttcggcgtcccaccaccccccaccacctccctcgtcgacacctacaggttcgtgcagagcgtcgccatcacatgccagaaagacgccgcccccgccgagaacaaagacccatacgacaaactgaaattctggaacgtcgacctgaaagagaaattcagcctggatctggaccagtacccattgggcaggaagttcctcgtccaggcgggtctccgtggcggtccgacgattggccctggctctcgttctgccccgtcggccacgaccagcagcggccctgccggtagcgtgggcgtggacgctggcaaataat

SEQ ID NO: 41 - DNA, 1573 bp, Artificial Sequence
  EXON (1)..(1573): 18L1DE137-138/59dES-mut4 nt
atggctctctggagaccctccgataacacagtgtacttgcccccccccagcgtcgcccgcgtcgtgaacacagacgactacgtcaccaggacctcaatcttctaccacgccggttcaagccgcctgctgaccgtcggcaacccctacttccgcgtccccgccggtggcggtaacaaacaagacatccccaaagtcagcgcctatcagtaccgcgtgttccgcgtccaactgcccgatcccaacaagttcggcctgcccgacacctccatctacaaccccgagacccagaggctggtctgggcatgcgccggcgtcgagatcggtaggggccaacccctgggcgtcggtttgtccggccaccccttctacaacaagctggacgataccgagtcctcccacgcagcaaccagcctgtacaagacctgcaagcaggccggtacctgcccctccgacgtcatcaacgtcagcgaagatgtccgcgataacgtcagcgtggactacaaacaaacccaactgtgcatcctcggttgcgcacccgccatcggcgagcattgggccaagggtaccgcctgcaagagcaggcccctgagccaaggtgactgtccacccctggagttgaagaataccgtcctcgaggacggcgacatggtggacaccggctacggcgcaatggatttctccaccctgcaggacaccaagtgcgaagtgcccctcgacatctgccaaagcatctgcaagtaccccgactacctgcagatgagcgccgacccctacggcgactccatgttcttctgtctgagaagggaacaattgttcgcccgccacttctggaaccgcgccggcaccatgggcgataccgtcccccagtccctgtacatcaagggtaccggcatgagggccagccccggttcatgcgtctacagcccaagcccctccggtagcatcgtcacaagcgattcccaactcttcaacaagccctactggctgcacaaagcccaaggccacaataacggcgtctgttggcacaaccagctgttcgtcaccgtcgtggacacaaccaggtccacaaacctgaccatctgcgccagcacccaaagccccgtgcccggccagtacgacgccacaaagttcaaacaatactcacgccacgtcgaagagtacgacctccaattcatcttccaactctgcaccatcaccctgaccgccgacgtcatgtcctacatccactccatgaactcatccatcctggaagactggaatttcggcgtcccaccaccccccaccacctccctcgtcgacacctacaggttcgtgcagagcgtcgccatcacatgccagaaagacgccgcccccgccgagaacaaagacccatacgacaaactgaaattctggaacgtcgacctgaaagagaaattcagcctggatctggaccagtacccattgggcaggaagttcctcgtccaggcgggtctccgtggcggtccgacgattggccctcgtggctcttctgccccgtcggccacgaccagcagcggccctgccgacagcgtgggcgtggacgctggcaaataat

SEQ ID NO: 42 - DNA, 1573 bp, Artificial Sequence
  EXON (1)..(1573): 18L1DE137-138/59dES-mut5 nt
atggctctctggagaccctccgataacacagtgtacttgcccccccccagcgtcgcccgcgtcgtgaacacagacgactacgtcaccaggacctcaatcttctaccacgccggttcaagccgcctgctgaccgtcggcaacccctacttccgcgtccccgccggtggcggtaacaaacaagacatccccaaagtcagcgcctatcagtaccgcgtgttccgcgtccaactgcccgatcccaacaagttcggcctgcccgacacctccatctacaaccccgagacccagaggctggtctgggcatgcgccggcgtcgagatcggtaggggccaacccctgggcgtcggtttgtccggccaccccttctacaacaagctggacgataccgagtcctcccacgcagcaaccagcctgtacaagacctgcaagcaggccggtacctgcccctccgacgtcatcaacgtcagcgaagatgtccgcgataacgtcagcgtggactacaaacaaacccaactgtgcatcctcggttgcgcacccgccatcggcgagcattgggccaagggtaccgcctgcaagagcaggcccctgagccaaggtgactgtccacccctggagttgaagaataccgtcctcgaggacggcgacatggtggacaccggctacggcgcaatggatttctccaccctgcaggacaccaagtgcgaagtgcccctcgacatctgccaaagcatctgcaagtaccccgactacctgcagatgagcgccgacccctacggcgactccatgttcttctgtctgagaagggaacaattgttcgcccgccacttctggaaccgcgccggcaccatgggcgataccgtcccccagtccctgtacatcaagggtaccggcatgagggccagccccggttcatgcgtctacagcccaagcccctccggtagcatcgtcacaagcgattcccaactcttcaacaagccctactggctgcacaaagcccaaggccacaataacggcgtctgttggcacaaccagctgttcgtcaccgtcgtggacacaaccaggtccacaaacctgaccatctgcgccagcacccaaagccccgtgcccggccagtacgacgccacaaagttcaaacaatactcacgccacgtcgaagagtacgacctccaattcatcttccaactctgcaccatcaccctgaccgccgacgtcatgtcctacatccactccatgaactcatccatcctggaagactggaatttcggcgtcccaccaccccccaccacctccctcgtcgacacctacaggttcgtgcagagcgtcgccatcacatgccagaaagacgccgcccccgccgagaacaaagacccatacgacaaactgaaattctggaacgtcgacctgaaagagaaattcagcctggatctggaccagtacccattgggcaggaagttcctcgtccaggcgggtctccgtggcaaaccgacgattggccctggctctcgttctgccccgtcggccacgaccagcagcggccctgccggtagcgtgagcgtgggcgctggcaaataat

SEQ ID NO: 43 - DNA, 1573 bp, Artificial Sequence
  EXON (1)..(1573): 18L1DE137-138/59dES-mut6 nt
atggctctctggagaccctccgataacacagtgtacttgcccccccccagcgtcgcccgcgtcgtgaacacagacgactacgtcaccaggacctcaatcttctaccacgccggttcaagccgcctgctgaccgtcggcaacccctacttccgcgtccccgccggtggcggtaacaaacaagacatccccaaagtcagcgcctatcagtaccgcgtgttccgcgtccaactgcccgatcccaacaagttcggcctgcccgacacctccatctacaaccccgagacccagaggctggtctgggcatgcgccggcgtcgagatcggtaggggccaacccctgggcgtcggtttgtccggccaccccttctacaacaagctggacgataccgagtcctcccacgcagcaaccagcctgtacaagacctgcaagcaggccggtacctgcccctccgacgtcatcaacgtcagcgaagatgtccgcgataacgtcagcgtggactacaaacaaacccaactgtgcatcctcggttgcgcacccgccatcggcgagcattgggccaagggtaccgcctgcaagagcaggcccctgagccaaggtgactgtccacccctggagttgaagaataccgtcctcgaggacggcgacatggtggacaccggctacggcgcaatggatttctccaccctgcaggacaccaagtgcgaagtgcccctcgacatctgccaaagcatctgcaagtaccccgactacctgcagatgagcgccgacccctacggcgactccatgttcttctgtctgagaagggaacaattgttcgcccgccacttctggaaccgcgccggcaccatgggcgataccgtcccccagtccctgtacatcaagggtaccggcatgagggccagccccggttcatgcgtctacagcccaagcccctccggtagcatcgtcacaagcgattcccaactcttcaacaagccctactggctgcacaaagcccaaggccacaataacggcgtctgttggcacaaccagctgttcgtcaccgtcgtggacacaaccaggtccacaaacctgaccatctgcgccagcacccaaagccccgtgcccggccagtacgacgccacaaagttcaaacaatactcacgccacgtcgaagagtacgacctccaattcatcttccaactctgcaccatcaccctgaccgccgacgtcatgtcctacatccactccatgaactcatccatcctggaagactggaatttcggcgtcccaccaccccccaccacctccctcgtcgacacctacaggttcgtgcagagcgtcgccatcacatgccagaaagacgccgcccccgccgagaacaaagacccatacgacaaactgaaattctggaacgtcgacctgaaagagaaattcagcctggatctggaccagtacccattgggcaggaagttcctcgtccaggcgggtctccgtggcaaaccgacgattggccctcgtggctcttctgccccgtcggccacgaccagcagcggccctgccggtagcgtgagcgtgggcgctggcaaataat

SEQ ID NO: 44 - protein, 23 aa, HPV 35
TQLYRTCKAAGTCPPDVIPKVEG

SEQ ID NO: 45 - protein, 23 aa, HPV 39
STLYRTCKQSGTCPPDVVDKVEG

SEQ ID NO: 46 - protein, 23 aa, HPV 51
TQLYSTCKAAGTCPPDVVNKVEG

SEQ ID NO: 47 - protein, 23 aa, HPV 53
TQLYQTCKQSGTCPEDVINKIEH

SEQ ID NO: 48 - protein, 23 aa, HPV 56
TQLYKTCKLSGTCPEDVVNKIEQ

SEQ ID NO: 49 - protein, 23 aa, HPV 59
LYKTCKQAGTCPSDVINKVEGTT

SEQ ID NO: 50 - protein, 23 aa, HPV 68
STLYKTCKQSGTCPPDVINKVEG

SEQ ID NO: 51 - protein, 23 aa, HPV 82
TQLYSTCKAAGTCPPDVIPKVKG